European Patent Specification EP 3 440 111 B1, published December 20, 2023. Title: anti-VEGFR-1 antibodies and uses thereof. Applicant: Fondazione Luigi Maria Monti Università degli Studi di Roma "Tor Vergata". The sequence listing filed with the application follows.

SEQUENCE LISTING (25 sequences)

SEQ ID NO: 1 - protein, 687 aa, Homo sapiens
MVSYWDTGVLLCALLSCLLLTGSSSGSKLKDPELSLKGTQHIMQAGQTLHLQCRGEAAHKWSLPEMVSKESERLSITKSACGRNGKQFCSTLTLNTAQANHTGFYSCKYLAVPTSKKKETESAIYIFISDTGRPFVEMYSEIPEIIHMTEGRELVIPCRVTSPNITVTLKKFPLDTLIPDGKRIIWDSRKGFIISNATYKEIGLLTCEATVNGHLYKTNYLTHRQTNTIIDVQISTPRPVKLLRGHTLVLNCTATTPLNTRVQMTWSYPDEKNKRASVRRRIDQSNSHANIFYSVLTIDKMQNKDKGLYTCRVRSGPSFKSVNTSVHIYDKAFITVKHRKQQVLETVAGKRSYRLSMKVKAFPSPEVVWLKDGLPATEKSARYLTRGYSLIIKDVTEEDAGNYTILLSIKQSNVFKNLTATLIVNVKPQIYEKAVSSFPDPALYPLGSRQILTCTAYGIPQPTIKWFWHPCNHNHSEARCDFCSNNEESFILDADSNMGNRIESITQRMAIIEGKNKMASTLVVADSRISGIYICIASNKVGTVGRNISFYITDVPNGFHVNLEKMPTEGEDLKLSCTVNKFLYRDVTWILLRTVNNRTMHYSISKQKMAITKEHSITLNLTIMNVSLQDSGTYACRARNVYTGEEILQKKEITIRGEHCNKKAVFSRISKFKSTRNDCTTQSNVKH

SEQ ID NO: 2 - protein, 13 aa, Artificial Sequence
  A4 peptide
TEGRELVIPARVT

SEQ ID NO: 3 - protein, 7 aa, Artificial Sequence
  B3 peptide
IPARVTS

SEQ ID NO: 4 - protein, 7 aa, Artificial Sequence
  ScrB3=S3 peptide
IARVSTP

SEQ ID NO: 5 - protein, 4 aa, Artificial Sequence
  C1 peptide
RVTS

SEQ ID NO: 6 - protein, 11 aa, Artificial Sequence
  A1 peptide
KFPLDTLIPDG

SEQ ID NO: 7 - protein, 11 aa, Artificial Sequence
  A2 peptide
DTLIPDGKRII

SEQ ID NO: 8 - protein, 10 aa, Artificial Sequence
  A3 peptide
GRPFVEMYSE

SEQ ID NO: 9 - protein, 12 aa, Artificial Sequence
  A5 peptide
DSRKGFIISNAT

SEQ ID NO: 10 - protein, 11 aa, Artificial Sequence
  A6 peptide
EATVNGHLYKT

SEQ ID NO: 11 - protein, 11 aa, Artificial Sequence
  A7 peptide
NITVTLKKFPL

SEQ ID NO: 12 - protein, 7 aa, Artificial Sequence
  P1 peptide
APARVTS

SEQ ID NO: 13 - protein, 7 aa, Artificial Sequence
  P2 peptide
IAARVTS

SEQ ID NO: 14 - protein, 7 aa, Artificial Sequence
  P3 peptide
IPAAVTS

SEQ ID NO: 15 - protein, 7 aa, Artificial Sequence
  P4 peptide
IPARATS

SEQ ID NO: 16 - protein, 7 aa, Artificial Sequence
  P5 peptide
IPARVAS

SEQ ID NO: 17 - protein, 7 aa, Artificial Sequence
  P6 peptide
IPARVTA

SEQ ID NO: 18 - DNA, 20 bp, Artificial Sequence
  primer
gcaccaagagcgatgtgtgg

SEQ ID NO: 19 - DNA, 20 bp, Artificial Sequence
  primer
acaccacggagttgtagtct

SEQ ID NO: 20 - DNA, 21 bp, Artificial Sequence
  primer
atttcccctgctcgtaccact

SEQ ID NO: 21 - DNA, 19 bp, Artificial Sequence
  primer
tcacgggtggggttcctca

SEQ ID NO: 22 - DNA, 399 bp, Artificial Sequence
  heavy chain D16F7
  CDS (1)..(399)
atgggatggagctctatcatcctcttcttggtagcaacagcctcaggtgtccactcccaggtccaactgcagcaacctgggtctgaactggtgaggcctggagcttcagtgaagctgtcctgcaaggcttctggctacatattcaccaactactggatgcactgggtgaagcagaggcctggacaaggccttgagtggattggagaaatttatcctcgtaatggtaatactaactacgatgagaagttcaagggcaaggccacactgactatagacacatcctccagcacagcctacatgcagctcagcagcctgacatctgaggactctgcggtctattactgtgccacctacctaggggactactggggccaaggcaccactctcacagtctcctca

SEQ ID NO: 23 - protein, 133 aa, Artificial Sequence
  Synthetic Construct
MGWSSIILFLVATASGVHSQVQLQQPGSELVRPGASVKLSCKASGYIFTNYWMHWVKQRPGQGLEWIGEIYPRNGNTNYDEKFKGKATLTIDTSSSTAYMQLSSLTSEDSAVYYCATYLGDYWGQGTTLTVSS

SEQ ID NO: 24 - DNA, 393 bp, Artificial Sequence
  D16F7 light chain
  CDS (1)..(393)
atgaagttgcctgttaggctgttggtgctgatgttctggattcctgcttccagcagtgatgttttgatgacccaaactccactctccctgcctgtcagccttggagatcaagcctccatctcttgcagatctagtcagagtattgttcatagtaatggaaacacctatttagaatggttcctgcagaaaccaggccagtctccaaagctcctgatctacaaagtttccaaccgattttctgggatcccagacaggttcagtggcagtggatcagggacagatttcacactcaagatcagtagagtggaggctgaggatctgggagtttatttctgctttcaaggttcacatgttccgtacacgttcggaggggggaccaagctggaaataaaa

SEQ ID NO: 25 - protein, 131 aa, Artificial Sequence
  Synthetic Construct
MKLPVRLLVLMFWIPASSSDVLMTQTPLSLPVSLGDQASISCRSSQSIVHSNGNTYLEWFLQKPGQSPKLLIYKVSNRFSGIPDRFSGSGSGTDFTLKISRVEAEDLGVYFCFQGSHVPYTFGGGTKLEIK